European Patent Application EP 4 806 986 A1, published September 16, 2026. Title: METHOD FOR PRODUCING CORNEAL ENDOTHELIAL CELLS. Applicant: OSAKA UNIVERSITY. The sequence listing filed with the application follows.

SEQUENCE LISTING (12 sequences)

SEQ ID NO: 1 - DNA, 21 bp, synthetic construct
  source 1..21: mol_type = other DNA
ttcctcccaaatcggtgactt

SEQ ID NO: 2 - DNA, 19 bp, synthetic construct
  source 1..19: mol_type = other DNA
cgccggtgttgacagacat

SEQ ID NO: 3 - DNA, 19 bp, synthetic construct
  source 1..19: mol_type = other DNA
gccaagggccttacatccg

SEQ ID NO: 4 - DNA, 20 bp, synthetic construct
  source 1..20: mol_type = other DNA
ggtggggaaaacatgctctg

SEQ ID NO: 5 - DNA, 21 bp, synthetic construct
  source 1..21: mol_type = other DNA
gactgtggcacctggataaga

SEQ ID NO: 6 - DNA, 21 bp, synthetic construct
  source 1..21: mol_type = other DNA
tcccactcagtgacatagcag

SEQ ID NO: 7 - DNA, 20 bp, synthetic construct
  source 1..20: mol_type = other DNA
gagccaggaatacgagggga

SEQ ID NO: 8 - DNA, 22 bp, synthetic construct
  source 1..22: mol_type = other DNA
tccagggatagtaatgcctgag

SEQ ID NO: 9 - DNA, 22 bp, synthetic construct
  source 1..22: mol_type = other DNA
agagtctgaagcaagagcactg

SEQ ID NO: 10 - DNA, 24 bp, synthetic construct
  source 1..24: mol_type = other DNA
tgcggtcatttatgttaaatcttc

SEQ ID NO: 11 - DNA, 21 bp, synthetic construct
  source 1..21: mol_type = other DNA
ggcgacacaggacaatcttta

SEQ ID NO: 12 - DNA, 19 bp, synthetic construct
  source 1..19: mol_type = other DNA
ggcagctccgttttcatgg